European Patent Specification EP 3 875 604 B1, published November 8, 2023. Title: New Fetal Methylation Markers. Applicant: The Chinese University of Hong Kong. Application EP. The sequence listing filed with the application follows.

SEQUENCE LISTING (38 sequences)

SEQ ID NO: 1 - DNA, 20 bp, Artificial Sequence
  methylation-specific PCR oligo Ras association (Ra1GDS/AF-6) domain family 1 (RASSF1A) RASSF1A-MF forward primer
gtgttaacgcgttgcgtatc

SEQ ID NO: 2 - DNA, 21 bp, Artificial Sequence
  methylation-specific PCR oligo Ras association (Ra1GDS/AF-6) domain family 1 (RASSF1A) RASSF1A-MR reverse primer
aaccccgcgaactaaaaacga

SEQ ID NO: 3 - DNA, 23 bp, Artificial Sequence
  methylation-specific PCR oligo Ras association (Ra1GDS/AF-6) domain family 1 (RASSF1A) RASSF1A-UF forward primer
tttggttggagtgtgttaatgtg

SEQ ID NO: 4 - DNA, 23 bp, Artificial Sequence
  methylation-specific PCR oligo Ras association (Ra1GDS/AF-6) domain family 1 (RASSF1A) RASSF1A-UR reverse primer
caaaccccacaaactaaaaacaa

SEQ ID NO: 5 - DNA, 30 bp, Artificial Sequence
  Ras association (Ra1GDS/AF-6) domain family 1 (RASSF1A) bisulfite sequencing oligo HsPromoter-F forward primer
gggttttatagtttttgtatttaggttttt

SEQ ID NO: 6 - DNA, 25 bp, Artificial Sequence
  Ras association (Ra1GDS/AF-6) domain family 1 (RASSF1A) bisulfite sequencing oligo HsPromoter-R reverse primer
caactcaataaactcaaactccccc

SEQ ID NO: 7 - DNA, 24 bp, Artificial Sequence
  Ras association (Ra1GDS/AF-6) domain family 1 (RASSF1A) bisulfite sequencing oligo HsExon1-F forward primer
ggggagtttgagtttattgagttg

SEQ ID NO: 8 - DNA, 22 bp, Artificial Sequence
  Ras association (Ra1GDS/AF-6) domain family 1 (RASSF1A) bisulfite sequencing oligo HsExon1-R reverse primer
ctaccccttaactaccccttcc

SEQ ID NO: 9 - DNA, 34 bp, Artificial Sequence
  adenomatosis polyposis coli (APC) bisulfite sequencing oligo HsPromoter-F forward primer
taatttatttaatattattgtttttttgtgttgt

SEQ ID NO: 10 - DNA, 26 bp, Artificial Sequence
  adenomatosis polyposis coli (APC) bisulfite sequencing oligo HsPromoter-R reverse primer
caccctaacraactacaccaatacaa

SEQ ID NO: 11 - DNA, 30 bp, Artificial Sequence
  retinoic acid receptor, beta (RARB) bisulfite sequencing oligo HsRARBPromoter-F forward primer
gtaggyggaatatygttttttaagttaagt

SEQ ID NO: 12 - DNA, 32 bp, Artificial Sequence
  retinoic acid receptor, beta (RARB) bisulfite sequencing oligo HsRARBPromoter-R reverse primer
acttcctactacttctatcacacaaaataaaa

SEQ ID NO: 13 - DNA, 32 bp, Artificial Sequence
  retinoic acid receptor, beta (RARB) bisulfite sequencing oligo HsRARBExon1-F forward primer
ttttattttgtgtgatagaagtagtaggaagt

SEQ ID NO: 14 - DNA, 28 bp, Artificial Sequence
  retinoic acid receptor, beta (RARB) bisulfite sequencing oligo HsRARBExon1-R reverse primer
aatcatttaccattttccaaacttactc

SEQ ID NO: 15 - DNA, 22 bp, Artificial Sequence
  methylation-specific PCR oligo caspase 8, apoptosis-related cysteine peptidase (CASP8) CASP8-MF forward primer
ggttaggggattcggagattgc

SEQ ID NO: 16 - DNA, 29 bp, Artificial Sequence
  methylation-specific PCR oligo caspase 8, apoptosis-related cysteine peptidase (CASP8) CASP8-MR reverse primer
aaaaaaaccgtatatctacattcgaaacg

SEQ ID NO: 17 - DNA, 25 bp, Artificial Sequence
  caspase 8, apoptosis-related cysteine peptidase (CASP8) bisulfite sequencing oligo HsExon1-F forward primer
agggaagtgtttttataggtttttt

SEQ ID NO: 18 - DNA, 29 bp, Artificial Sequence
  caspase 8, apoptosis-related cysteine peptidase (CASP8) bisulfite sequencing oligo HsExon1-R reverse primer
ataatttcctattaaaaaaaccaccttaa

SEQ ID NO: 19 - DNA, 21 bp, Artificial Sequence
  methylation-specific PCR oligo secretoglobulin, family 3A, member 1 (SCGB3A1) SCGB3A1-MF forward primer
tttagttttgtaggggggcgc

SEQ ID NO: 20 - DNA, 24 bp, Artificial Sequence
  methylation-specific PCR oligo secretoglobulin, family 3A, member 1 (SCGB3A1) SCGB3A1-MF forward primer
accaacttcctactacgaccgacg

SEQ ID NO: 21 - DNA, 25 bp, Artificial Sequence
  secretoglobulin, family 3A, member 1 (SCGB3A1) bisulfite sequencing oligo Hspromoter-F forward primer
gattagaggtagggattagggagtt

SEQ ID NO: 22 - DNA, 24 bp, Artificial Sequence
  secretoglobulin, family 3A, member 1 (SCGB3A1) bisulfite sequencing oligo Hspromoter-R reverse primer
taacaaacrctaaaaccctctaaa

SEQ ID NO: 23 - DNA, 19 bp, Artificial Sequence
  methylation-specific PCR oligo DOC-2/DAB2 interacting protein (DAB2IP) DAB2IP-MF forward primer
gtaagggtgcgggtttcgc

SEQ ID NO: 24 - DNA, 23 bp, Artificial Sequence
  methylation-specific PCR oligo DOC-2/DAB2 interacting protein (DAB2IP) DAB2IP-MR reverse primer
gaactcacctctcattatccgcg

SEQ ID NO: 25 - DNA, 28 bp, Artificial Sequence
  DOC-2/DAB2 interacting protein (DAB2IP) bisulfite sequencing oligo HsExon1-F forward primer
aagggttttattaagygtattaagagtt

SEQ ID NO: 26 - DNA, 20 bp, Artificial Sequence
  DOC-2/DAB2 interacting protein (DAB2IP) bisulfite sequencing oligo HsExon1-R reverse primer
accccraaaaaaaacacaaa

SEQ ID NO: 27 - DNA, 20 bp, Artificial Sequence
  RASSF1A real-time PCR forward primer RSF-b151F
agcctgagctcattgagctg

SEQ ID NO: 28 - DNA, 16 bp, Artificial Sequence
  RASSF1A real-time PCR reverse primer RSF-dsgnR
accagctgccgtgtgg

SEQ ID NO: 29 - DNA, 16 bp, Artificial Sequence
  RASSF1A real-time PCR minor groove binding (MGB) fluorescent probe RSF-dsgnT
  modified_base (1)...(1): n = c modified by FAM
  modified_base (16)...(16): n = t modified by minor groove binder (MGB)
ncaacgcgctgcgcan

SEQ ID NO: 30 - DNA, 17 bp, Artificial Sequence
  beta-actin real-time PCR forward primer Actin-163F
gcgccgttccgaaagtt

SEQ ID NO: 31 - DNA, 15 bp, Artificial Sequence
  beta-actin real-time PCR reverse primer Actin-298R
cggcggatcggcaaa

SEQ ID NO: 32 - DNA, 17 bp, Artificial Sequence
  beta-actin real-time PCR minor groove binding (MGB) fluorescent probe Actin-243T
  modified_base (1)...(1): n = a modified by VIC
  modified_base (17)...(17): n = c modified by minor groove binder (MGB)
nccgccgagaccgcgtn

SEQ ID NO: 33 - DNA, 21 bp, Artificial Sequence
  Y-chromosome sex-determining region Y (SRY) real-time PCR forward amplification primer SRY-109F
tggcgattaagtcaaattcgc

SEQ ID NO: 34 - DNA, 25 bp, Artificial Sequence
  Y-chromosome sex-determining region Y (SRY) real-time PCR reverse amplification primer SRY-245R
ccccctagtaccctgacaatgtatt

SEQ ID NO: 35 - DNA, 26 bp, Artificial Sequence
  Y-chromosome sex-determining region Y (SRY) real-time PCR minor groove binding (MGB) fluorescent probe SRY-142T
  modified_base (1)...(1): n = a modified by FAM
  modified_base (26)...(26): n = a modified by TAMRA
ngcagtagagcagtcagggaggcagn

SEQ ID NO: 36 - DNA, 16 bp, Artificial Sequence
  RASSF1A extension primer Rsf-R17
cagccgggtgggccct

SEQ ID NO: 37 - DNA, 17 bp, Artificial Sequence
  RASSF1A genotype A primer extension reaction product
  modified_base (17)...(17): n = dideoxythymidine
cagccgggtgggccctn

SEQ ID NO: 38 - DNA, 18 bp, Artificial Sequence
  RASSF1A genotype C primer extension reaction product
  modified_base (18)...(18): n = dideoxycytidine
cagccgggtgggccctgn